European Patent Specification EP 3 580 353 B1, published September 13, 2023. Title: PROBE COMBINATION FOR DETECTION OF CANCER. Applicant: TCM BIOTECH INTERNATIONAL CORP. The sequence listing filed with the application follows.

SEQUENCE LISTING (56 sequences)

SEQ ID NO: 1 - DNA, 3191 bp, Hepatitis B virus
ctccaccactttccaccaaactcttcaagatcccagagtcagggccctgtactttcctgctggtggctccagttcaggaacagtgagccctgctcagaatactgtctctgccatatcgtcaatcttatcgaagactggggaccctgtaccgaacatggagaacatcgcatcaggactcctaggacccctgctcgtgttacaggcggggtttttcttgttgacaaaaatcctcacaataccacagagtctagactcgtggtggacttctctcaattttctagggggaacacccgtgtgtcttggccaaaattcgcagtcccaaatctccagtcactcaccaacctgttgtcctccaatttgtcctggttatcgctggatgtgtctgcggcgttttatcatcttcctctgcatcctgctgctatgcctcatcttcttgttggttcttctggactatcaaggtatgttgcccgtttgtcctctaattccaggatcatcaacaaccagcaccggaccatgcaaaacctgcacaactcctgctcaaggaacctctatgtttccctcatgttgctgtacaaaacctacggacggaaactgcacctgtattcccatcccatcatcttgggctttcgcaaaatacctatgggagtgggcctcagtccgtttctcttggctcagtttactagtgccatttgttcagtggttcgtagggctttcccccactgtctggctttcagttatatggatgatgtggtattgggggccaagtctgtacaacatcttgagtccctttatgccgctgttaccaattttcttttgtctttgggtatacatttaaaccctcacaaaacaaaaagatggggatattcccttaacttcatgggatatgtaattgggagttggggcacattgccacaggaacatattgtacaaaaaatcaaaatgtgttttaggaaacttcctgtaaacaggcctattgattggaaagtatgtcaacgaattgtgggtcttttggggtttgccgcccctttcacgcaatgtggatatcctgctttaatgcctttatatgcatgtatacaagcaaaacaggcttttactttctcgccaacttacaaggcctttctaagtaaacagtatctgaacctttaccccgttgctcggcaacggcctggtctgtgccaagtgtttgctgacgcaacccccactggttggggcttggccataggccatcagcgcatgcgtggaacctttgtgtctcctctgccgatccatactgcggaactcctagccgcttgttttgctcgcagcaggtctggagcaaaactcatcgggactgacaattctgtcgtgctctcccgcaagtatacatcatttccatggctgctaggctgtgctgccaactggatcctgcgcgggacgtcctttgtttacgtcccgtcggcgctgaatcccgcggacgacccctcccggggccgcttggggctctaccgcccgcttctccgcctgttgtaccgaccgaccacggggcgcacctctctttacgcggactccccgtctgtgccttctcatctgccggaccgtgtgcacttcgcttcacctctgcacgtcgcatggagaccaccgtgaacgcccaccggaacctgcccaaggtcttgcataagaggactcttggactttcagcaatgtcaacgaccgaccttgaggcatacttcaaagactgtgtgtttactgagtgggaggagttgggggaggagattaggttaaaggtctttgtactaggaggctgtaggcataaattggtgtgttcaccagcaccatgcaactttttcacctctgcctaatcatctcatgttcatgtcctactgttcaagcctccaagctgtgccttgggtggctttggggcatggacattgacccgtataaagaatttggagcttctgtggagttactctcttttttgccttctgacttctttccttctattcgagatctcctcgacaccgcctctgctctgtatcgggaggccttagagtctccggaacattgttcacctcaccatacggcactcaggcaagctattctgtgttggggtgagttaatgaatctagccacctgggtgggaagtaatttggaagatccagcatccagggaattagtagtcagctatgtcaacgttaatatgggcctaaaaatcagacaactattgtggtttcacatttcctgtcttacttttggaagagaaactgttcttgaatatttggtgtcttttggagtgtggattcgcactcctcctgcatatagaccaccaaatgcccctatcttatcaacacttccggaaactactgttgttagacgaagaggcaggtcccctagaagaagaactccctcgcctcgcagacgaaggtctcaatcgccgcgtcgcagaagatctcaatctcgggaatctcaatgttagtattccttggacacataaggtgggaaactttacggggctttattcttctacggtaccttgctttaatcctaaatggcaaactccttcttttcctgacattcatttgcaggaggacattgttgatagatgtaagcaatttgtggggccccttacagtaaatgaaaacaggagactaaaattaattatgcctgctaggttttatcccaatgttactaaatatttgcccttagataaagggatcaaaccttattatccagagcatgtagttaatcattacttccagacgagacattatttacacactctttggaaggcgggtatcttatataaaagagagtccacacgtagcgcctcattttgcgggtcaccatattcttgggaacaagatctacagcatgggaggttggtcttccaaacctcgaaaaggcatggggacaaatctttctgtccccaatcccctgggattcttccccgatcatcagttggaccctgcattcaaagccaactcagaaaatccagattgggacctcaacccgcacaaggacaactggccggacgccaacaaggtgggagtgggagcattcgggccagggttcacccctccccatgggggactgttggggtggagccctcaggctcagggcatactcacaactgtgccagcagctcctcctcctgcctccaccaatcggcagtcaggaaggcagcctactcccttatctccacctctaagggacac

SEQ ID NO: 2 - DNA, 3191 bp, Hepatitis B virus
ctccacaacattccaccaagctctgctagatcccagagtgaggggcctatactttcctgctggtggctccagttccggaacagtaaaccctgttccgactactgcctcacccatatcgtcaatcttctcgaggactggggaccctgcaccgaacatggagaacacaacatcaggattcctaggacccctgctcgtgttacaggcggggtttttcttgttgacaagaatcctcacaataccacagagtctagactcgtggtggacttctctcaattttctagggggagcacccacgtgtcctggccaaaattcgcagtccccaacctccaatcactcaccaacctcttgtcctccaatttgtcctggctatcgctggatgtgtctgcggcgttttatcatattcctcttcatcctgctgctatgcctcatcttcttgttggttcttctggactaccaaggtatgttgcccgtttgtcctctacttccaggaacatcaactaccagcacgggaccatgcaagacctgcacgattcctgctcaaggaacctctatgtttccctcttgttgctgtacaaaaccttcggacggaaactgcacttgtattcccatcccatcatcctgggctttcgcaagattcctatgggagtgggcctcagtccgtttctcctggctcagtttactagtgccatttgttcagtggttcgtagggctttcccccactgtttggctttcagttatatggatgatgtggtattgggggccaagtctgtacaacatcttgagtccctttttacctctattaccaattttcttttgtctttgggtatacatttgaaccctaataaaaccaaacgttggggctactcccttaacttcatgggatatgtaattggaagttggggtactttaccacaggaacatattgtactaaaaatcaagcaatgttttcgaaaactgcctgtaaatagacctattgattggaaagtatgtcaaagaattgtgggtcttttgggctttgctgccccttttacacaatgtggctatcctgccttaatgcctttatatgcatgtatacaatctaagcaggctttcactttctcgccaacttacaaggcctttctgtgtaaacaatatctgaacctttaccccgttgcccggcaacggtcaggtctctgccaagtgtttgctgacgcaacccccactggatggggcttggccataggccatcggcgcatgcgtggaacctttgtggctcctctgccgatccatactgcggaactcctagcagcttgttttgctcgcagccggtctggagcgaaacttatcggcaccgacaactctgttgtcctctctcggaaatacacctcctttccatggctgctagggtgtgctgccaactggatcctgcgcgggacgtcctttgtctacgtcccgtcggcgctgaatcccgcggacgacccgtctcggggccgtttgggactctaccgtccccttcttcatctgccgttccggccgaccacggggcgcacctctctttacgcggtctccccgtctgtgccttctcatctgccggaccgtgtgcacttcgcttcacctctgcacgtcgcatggagaccaccgtgaacgcccaccaggtcttgcccaaggtcttacataagaggactcttggactctcagcaatgtcaacgaccgaccttgaggcatacttcaaagactgtttgtttaaagactgggaggagttgggggaggagattaggttaatgatctttgtactaggaggctgtaggcataaattggtctgttcaccagcaccatgcaactttttcacctctgcctaatcatctcatgttcatgtcctactgttcaagcctccaagctgtgccttgggtggctttggggcatggacattgacccgtataaagaatttggagcttctgtggagttactctcttttttgccttctgacttctttccttctattcgagatctcctcgacaccgcctctgctctgtatcgggaggccttagagtctccggaacattgttcacctcaccatacagcactcaggcaagctattctgtgttggggtgagttgatgaatctggccacctgggtgggaagtaatttggaagacccagcatccagggaattagtagtcagctatgtcaatgttaatatgggcctaaaaatcagacaactattgtggtttcacatttcctgtcttacttttggaagagaaactgttcttgagtatttggtgtcttttggagtgtggattcgcactcctcccgcttacagaccaccaaatgcccctatcttatcaacacttccggaaactactgttgttagacgacgaggcaggtcccctagaagaagaactccctcgcctcgcagacgaaggtctcaatcgccgcgtcgcagaagatctcaatctcgggaatctcaatgttagtatcccttggactcataaggtgggaaactttactgggctttattcttctactgtacctgtctttaatcctgagtggcaaactccctcctttcctcacattcatttacaggaggacattattaatagatgtcaacaatatgtgggccctcttacagttaatgaaaaaaggagattaaaattaattatgcctgctaggttctatcctaaccttaccaaatatttgcccttggataaaggcattaaaccttattatcctgaacatgcagttaatcattacttcaaaactaggcattatttacatactctgtggaaggctggcattctatataagagagaaactacacgcagcgcctcattttgtgggtcaccatattcttgggaacaagagctacagcatgggaggttggtcttccaaacctcgacaaggcatggggacgaatctttctgttcccaatcctctgggattctttcccgatcaccagttggaccctgcgttcggagccaactcaaacaatccagattgggacttcaaccccaacaaggatcactggccagaggcaaatcaggtaggagcgggagcattcgggccagggttcaccccaccacacggcggtcttttggggtggagccctcaggctcagggcatattgacaacagtgccagcagcacctcctcctgcctccaccaatcggcagtcaggaagacagcctactcccatctctccacctctaagagaaag

SEQ ID NO: 3 - DNA, 960 bp, Hepatitis B virus
cgcatgcgtggaacctttgtggctcctctgccgatccatactgcggaactcctagccgcttgttttgctcgcagccggtctggagcaaagctcatcggaactgacaattctgtcgtcctctcgcggaaatatacatcgtttccatggctgctaggctgtgctgccaactggatccttcgcggaacgtcctttgtctacgtcccgtcggcgctgaatcccgcggacgacccctctcggggccgcttgggactctctcgtccccttctccgtctgccgttccagccgaccacggggcgcacctctctttacgcggtctccccgtctgtgccttctcatctgccggtccgtgtgcacttcgcttcacctctgcacgttgcatggagaccaccgtgaacgcccatcagatcctgcccaaggtcttacataagaggactcttggactcccagcaatgtcaacgaccgaccttgaggcctacttcaaagactgtgtgtttaaggactgggaggagctgggggaggagattaggttaaaggtctttgtattaggaggctgtaggcataaattggtctgcgcaccagcaccatgcaactttttcacctctgcctaatcatctcttgtacatgtcccactgttcaagcctccaagctgtgccttgggtggctttggggcatggacattgacccttataaagaatttggagctactgtggagttactctcgtttttgccttctgacttctttccttccgtcagagatctcctagacaccgcctcagctctgtatcgagaagccttagagtctcctgagcattgctcacctcaccatactgcactcaggcaagccattctctgctggggggaattgatgactctagctacctgggtgggtaataatttggaagatccagcatccagggatctagtagtcaattatgttaatactaacatgggtttaaagat

SEQ ID NO: 4 - DNA, 960 bp, Hepatitis B virus
cgcatgcgtggaacctttgtggctcctctgccgatccatactgcggaactcctagccgcttgttttgctcgcagccggtctggagcaaagctcatcggaactgacaattctgtcgtcctctcgcggaaatatacatcgtttccatggctgctaggctgtactgccaactggatccttcgcgggacgtcctttgtttacgtcccgtcggcgctgaatcccgcggacgacccctctcggggccgcttgggactctctcgtccccttctccgtctgccgttccagccgaccacggggcgcacctctctttacgcggtctccccgtctgtgccttctcatctgccggtccgtgtgcacttcgcttcacctctgcacgttgcatggagaccaccgtgaacgcccatcagatcctgcccaaggtcttacataagaggactcttggactcccagcaatgtcaacgaccgaccttgaggcctacttcaaagactgtgtgtttaaggactgggaggagctgggggaggagattaggttaatgatctttgtattaggaggctgtaggcataaattggtctgcgcaccagcaccatgcaactttttcacctctgcctaatcatctcttgtacatgtcccactgttcaagcctccaagctgtgccttgggtggctttggggcatggacattgacccttataaagaatttggagctactgtggagttactctcgtttttgccttctgacttctttccttccgtcagagatctcctagacaccgcctcagctctgtatcgagaagccttagagtctcctgagcattgctcacctcaccatactgcactcaggcaagccattctctgctggggggaattgatgactctagctacctgggtgggtaataatttggaagatccagcatccagggatctagtagtcaattatgttaatactaacatgggtttaaagat

SEQ ID NO: 5 - DNA, 960 bp, Hepatitis B virus
cgcatgcgtggaacctttgtggctcctctgccgatccatactgcggaactcctagccgcttgttttgctcgcagccggtctggagcaaaactcatcgggactgacaattctgtcgtcctttctcggaaatatacatccttcccatggctgctaggttgtactgccaactggattcttcgagggacgtcctttgtctacgtcccgtcggcgctgaatcccgcggacgacccctcgcgaggtcgcttgggactctatcgtccccttctccgtctgccgtaccgtccgaccacggggcgcacctctctttacgcggtctccccgtctgtgccttctcatctgccggtccgtgtgcacttcgcttcacctctgcacgttgcatggagaccaccgtgaacgcccatcagatcctgcccaaggtcttatataagaggactcttggactcccagcaatgtcaacgaccgaccttgaggcctacttcaaagactgtgtgtttaaagactgggaggagttgggggaggagattaggttaaaggtttatgtattaggaggctgtaggcataaattggtctgcgcaccatcatcatgcaactttttcacctctgcctaatcatctcttgtacatgtcccacttttcaagcctccaagctgtgccttgggtggctttggggcatggacattgacccttataaagaatttggagctacagtggagttactctcgtttttgccttctgacttctttccttccgtccgggatctactagatacagcctcagctctgtatcgggaagcattagagtctcctgagcattgctcacctcaccatacagcactcaggcaagccattctctgctggggggatgtactggatctatctacctgggtgggtgctaatttgcaagatccagcatccagggatctagtagtcaattatgttaatactaacatgggcctaaagtt

SEQ ID NO: 6 - DNA, 960 bp, Hepatitis B virus
cgcatgcgtggaacctttgtgtctcctctgccgatccatactgcggaactcctagccgcttgttttgctcgcagcaggtctggggcaaaactcatcgggactgacaattctgtcgtgctctcccgcaagtatacatcgttcccatggctgctaggctgtgctgccaactggatcctgcgcgggacgtcctttgtttacgtcccgtcggcgctgaatcccgcggacgacccctcccggggccgcttggggctctaccgcccgcttctccgcctgttgtaccgtccgaccacggggcgcacctctctttacgcggactccccgtctgtgccttctcatctrccggaccgtgtgcacttcgcttcacctctgcacgtcgcatggagaccaccgtgaacgcccaccggaacctgcccaaggtcttgcataagaggactcttggactttcmgcaatgtcaacgaccgaccttgaggcatacttcaaagactgtgtgtttaatgagtgggaggagttgggggaggagaktaggttaaaggtctttgtactaggaggctgtaggcataaattggtgygttcaccagcaccatgcaactttttcacctctgcctaatcatctcatgttcatgtcctactgttcaagcctccaagctgtgccttgggtggctttagggcatggacattgacccgtataaagaatttggagcttctgtggagttactctcttttttgcctcatgacttctttccttctattcgagatctcctcgacaccgcctctgctttgtatcgggaggccttagagtctccggaacattgttcacctcaccatacggcactcaggcaagctattctgtgttggggtgagttgatgaatctagccacctgggtgggaagtaatttggaagatccagcatccagggaattagtcgttagctatgtcaacgttaatatgggcmtaaaaat

SEQ ID NO: 7 - DNA, 960 bp, Hepatitis B virus
cgcatgcgtggaacctttgtgtctcctctgccgatccatactgcggaactcctagccgcttgttttgctcgcagcaggtctggagcgaaactcatcgggactgacaattctgtcgtgctctcccgcaagtatacatcgtttccatggctgctaggctgtgctgccaactggatcctgcgcgggacgtcctttgtttacgtcccgtcggcgctgaatcccgcggacgacccctcccggggccgcttggggctctaccgcccgcttctccgtctgccgtaccgaccgaccacggggcgcacctctctttacgcggactccccgtctgtgccttctcgtctgccggaccgtgtgcacttcgcttcacctctgcacgtcgcatggaaaccaccgtgaacgcccaccggaacctgcccaaggtcttgcacaagaggactcttggactttcagcaatgtcaacgaccgaccttgaggcatacttcaaagactgtgtgtttcatgagtgggaggagctgggggaggagattaggttaaaggtctttgtactaggaggctgtaggcataaattggtctgttcaccagcaccatgcaactttttcacctctgcctagtcatctcttgttcatgtcctactgttcaagcctccaagctgtgccttgggtggctttgggacatggacattgacccttataaagaatttggagctactgtggagttactctcttttttgccttctgacttctttccgtcggtacgagacctcctagataccgctgctgctctgtatcgggaagccttagaatctcctgaacattgctcacctcaccacacagcactcaggcaagctattctgtgctggggggaattaatgactctagctacctgggtgggtaataatttagaagatccagcgtccagggatctagtagtcaattatgttaacactaacatgggcctaaagat

SEQ ID NO: 8 - DNA, 960 bp, Hepatitis B virus
cgcatgcgtgggacctttgtgtctcctctgccgatccatactgcggaactcctagccgcttgttttgctcgcagcaggtctggagcgaaacttatcgggactgacaattccgttgtcctttcccgcaaatatacatcgtttccatggctgctaggctgtgctgccaactggatcctgcgcgggacgtcctttgtctacgtcccgtcggcgctgaatcccgcggacgacccctcccggggccgcttggggctctaccgcccgcttctccgtctgccgtaccgaccgaccacggggcgcacctctctttacgcggactccccgtctgtgccttctcgtctgccggaccgtgtgcacttcgcttcacctctgcacgtcgcatggagaccaccgtgaacgcccaccggaacttgcccaaggtcttgcataagaggactcttggactttcagcaatgtcaacgaccgaccttgaggcatacttcaaagactgtgtgtttaatgagtgggaggagttgggggaggagattaggttaaaggtctttgtactaggaggctgtaggcataaattggtctgttcaccagcaccatgcaactttttcacctctgcctaatcatctcatgttcatgtcctactgttcaagcctccaagctgtgccttgggtggctttggggcatggacattgacccgtataaagaatttggagcttctgtggagttactctcttttttgccttctgacttctttccttctattcgagatcttctcgacaccgcctctgctctgtatcgggaggccttagagtctccggaacattgttcacctcaccatacggcactcaggcaagctattctgtgttggggtgagttaatgaatctagccacctgggtgggaagtaatttggaagacccagcatccagggaattagtagtcagctatgtcaatgttaatatgggcctaaaaat

SEQ ID NO: 9 - DNA, 960 bp, Hepatitis B virus
cgcatgcgtggaacctttgtgtctcctctgccgatccatactgcggaactcctagccgcttgttttgctcgcagcaggtctggagcaaaactcatcgggactgacaattctgtcgtgctctcccgcaagtatacatcatttccatggctgctaggctgtgctgccaactggatcctgcgcgggacgtcctttgtttacgtcccgtcggcgctgaatcccgcggacgacccctcccggggccgcttggggctctaccgcccgcttctccgcctgttgtaccgaccgaccacggggcgcacctctctttacgcggactccccgtctgtgccttctcatctgccggaccgtgtgcacttcgcttcacctctgcacgtcgcatggagaccaccgtgaacgcccaccggaacctgcccaaggtcttgcataagaggactcttggactttcagcaatgtcaacgaccgaccttgaggcatacttcaaagactgtgtgtttactgagtgggaggagttgggggaggagattaggttaaaggtctttgtactaggaggctgtaggcataaattggtgtgttcaccagcaccatgcaactttttcacctctgcctaatcatctcatgttcatgtcctactgttcaagcctccaagctgtgccttgggtggctttggggcatggacattgacccgtataaagaatttggagcttctgtggagttactctcttttttgccttctgacttctttccttctattcgagatctcctcgacaccgcctctgctctgtatcgggaggccttagagtctccggaacattgttcacctcaccatacggcactcaggcaagctattctgtgttggggtgagttaatgaatctagccacctgggtgggaagtaatttggaagatccagcatccagggaattagtagtcagctatgtcaacgttaatatgggcctaaaaat

SEQ ID NO: 10 - DNA, 960 bp, Hepatitis B virus
cgcatgcgtggaacctttgtggctcctctgccgatccatactgcggaactcctagcagcttgttttgctcgcagccggtctggagctaaacttatcgggactgacaactctgttgtcctctcgcggaaatacacctccttcccatggctgctcgggtgtgctgccaactggatcctgcgcgggacgtcctttgtctacgtcccgtcggcgctgaatcccgcggacgacccatctcggggccgtttgggcctctaccgtccccttcttcacctgccgttccagccgaccacggggcgcacctctctttacgcggactccccgtctgtgccttctcatctgccggaccgtgtgcacttcgcttcacctctgcacgtcgcatggagaccaccgtgaacgcccaccaggtcttgcccaagctcttacataagaggactcttggactctcagcaatgtcaacgaccgaccttgaggcatacttcaaagactgtttgtttaaagactgggaggagttgggggaggagattaggttaaaggtctttgtactaggaggctgtaggcataaattggtctgttcaccagcaccatgcaactttttcccctctgcctaatcatctcatgttcatgtcctactgttcaagcctccaagctgtgccttgggtggctttggggcatggacattgacccgtataaagaatttggagcttctgtggagttactctcttttttgccttctgacttctttccttctattcgagatctcctcgataccgcctctgctctgtatcgggaggccttagagtctccggaacattgttcacctcaccatacagcactcaggcaagctattctgtgttggggtgagttgatgaatctggccacctgggtgggaagtaatttggaagacccagcatccagggaattagtagtcagctatgtcaatgttaatatgggcctaaaaat

SEQ ID NO: 11 - DNA, 961 bp, Hepatitis B virus
cgcatgcgtggaacctttgtggctcctctgccgatccatactgcggaactcctagcggcttwgttttgctcgcagccggtctggagcgaacctcatcggcaccgacaactctgttgtcctctctcggaagtacacctcctttccatggctgctaggatgtgctgccaactggatcctgcgcgggacgtcctttgtctacgtcccgtcggcgctgaatcccgcggacgacccctctcggggccgcttggggatctaccgtcccctcctccgtctgccgttccggccgaccacggggcgcacctctctttacgcggtctccccgtctgtgccttctcatctgccggaccgtgtgcacttcgcttcacctctgcacgtcgcatggagaccaccgtgaacgcccaccaggtcttgcccaaggtcttgcataagaggactcttggactctcagcaatgtcaacgaccgaccttgaggcatacttcaaagactgtgtgtttaaagactgggaggagttgggggaggagattaggttaaaggtctttgtactaggaggctgtaggcataaattggtctgttcaccagcaccatgcaactttttcacctctgcctaatcatctcatgttcatgtcctactgttcaagcctccaagctgtgccttgggtggctttggggcatggacattgacccttataaagaatttggagcttctgtggagttactctcttttttgccgtctgatttctttccatctattcgagatctcctagacactgcctcagctctgtatcgggaagccttagagtctccggaacattgttcacctcaccatacagcactcaggcaagctgttctgtgttggggtgaattaatgaatctggctacctgggtgggaagtaatttggaagatccagcatccagggaattagtagtcagttatgtcaatgttaatatgggcttaaagat

SEQ ID NO: 12 - DNA, 960 bp, Hepatitis B virus
cgcatgcgtggaacctttgtggctcctctgccgatccatactgcggaactcctggcagcttgttttgctcgcagccggtctggagcgaaacttatcgggactgacaactctgttgtcctttctcggaaatacacctccttcccatggctgctcggatgtgctgccaactggatcctgcgcgggacgtcctttgtctacgtcccgtcggcgctgaatcccgcggacgacccgtctcggggccgtttgggcctctaccgtccccttctgcagctgccgttccggccgaccacggggcgcacctctctttacgcggtctccccgtctgtgccttctcatctgccggaccgtgtgcacttcgcttcacctctgcacgtcgcatggagaccaccgtgaacgcccaccaggtcttgcccaaggtcttacataagaggactcttggactctcagcaatgtcaacgaccgaccttgaggcatacttcaaagactgtttgtttaaagactgggaggagttgggggaggagattaggttaaaggtctttgtactaggaggctgtaggcataaattggtctgttcaccagcaccatgcaactttttcacctctgcctaatcatctcatgttcatgtcccactgttcaagcctccaagctgtgccttgggtggctttggggcatggacattgacccgtataaagaatttggagcttctgtggagttactctcttttttgccttctgacttctttccttctattcgagatctcctcgacaccgcctctgcactgtatcgggaggccttagagtctccggaacattgttcacctcaccatacagcactcaggcaagctattctgtgttggggtgagttgatgaatctggccacctgggtgggaagtaatttggaagacccagcatccagggaattagtagtcagctatgtcaatgttaacatgggcctaaaaat

SEQ ID NO: 13 - DNA, 960 bp, Hepatitis B virus
cgcatgcgtggaacctttgtggctcctctgccgatccatactgcggaactcctagcagcttgttttgctcgcagccggtctggagcgaaacttatcggcaccgacaactctgttgtcctctctcggaaatacacctcctttccatggctgctagggtgtgctgccaactggatcctgcgcgggacgtcctttgtctacgtcccgtcggcgctgaatcccgcggacgacccgtctcggggccgtttgggactctaccgtccccttcttcatctgccgttccggccgaccacggggcgcacctctctttacgcggtctccccgtctgtgccttctcatctgccggaccgtgtgcacttcgcttcacctctgcacgtcgcatggagaccaccgtgaacgcccaccaggtcttgcccaaggtcttacataagaggactcttggactctcagcaatgtcaacgaccgaccttgaggcatacttcaaagactgtttgtttaaagactgggaggagttgggggaggagattaggttaatgatctttgtactaggaggctgtaggcataaattggtctgttcaccagcaccatgcaactttttcacctctgcctaatcatctcatgttcatgtcctactgttcaagcctccaagctgtgccttgggtggctttggggcatggacattgacccgtataaagaatttggagcttctgtggagttactctcttttttgccttctgacttctttccttctattcgagatctcctcgacaccgcctctgctctgtatcgggaggccttagagtctccggaacattgttcacctcaccatacagcactcaggcaagctattctgtgttggggtgagttgatgaatctggccacctgggtgggaagtaatttggaagacccagcatccagggaattagtagtcagctatgtcaatgttaatatgggcctaaaaat

SEQ ID NO: 14 - DNA, 960 bp, Hepatitis B virus
cgcgtgcgtggaaccttttcggctcctctgccgatccatactgcggaactcctagccgcttgttttgctcgcagcaggtctggagcaaacattatcgggactgataactctgttgtcctctcccgcaaatatacatcgtatccatggctgctaggctgtgctgccaactggatcctgcgcgggacgtcctttgtttacgtcccgtcggcgctgaatcctgcggacgacccttctcggggtcgcttgagactctctcgtccccttctccgtctgccgttccgaccgaccacggggcgcacctctctttacgcggactccccgtctgtgccttctcatctgccggaccgtgtgcacttcgcttcacctctgcacgtcgcatggagaccaccgtgaacgcccaccgaatgttgcccaaggtcttacataagaggactcttggactctctgcaatgtcaacgaccgaccttgaggcatacttcaaagactgtttgtttaaagactgggaggagttgggggaggagattagattaaaggtctttgtactaggaggctgtaggcataaattggtctgcgcaccggcgccatgcacctttttcacctctgcctaatcatctcttgttcatgtcctactgttcaagcctccaagctgtgccttgggtggctttggggcatggacatcgacccttataaagaatttggagctactgtggagttactctcgtttttgccttctgacttctttccttcagtacgagatcttctagataccgcctcagctctgtatcgggaagccttagagtctcctgagcattgttcacctcaccatactgcactcaggcaagcaattctttgctggggggaactaatgactctagctacctgggtgggtgttaatttggaagatccagcatctagagacctagtagtcagttatgtcaacactaatatgggcctaaagtt

SEQ ID NO: 15 - DNA, 960 bp, Hepatitis B virus
cgcatgcgtggaacctttttggctcctctgccgatccatactgcggaactcctagccgcttgttttgctcgcagcaggtctggagcaaacattctcgggactgacaactctgttgtcctctcccgcaaatatacatcgtttccatggctgctaggctgtgctgccaactggatcctgcgcgggacgtcctttgtttacgtcccgtcgrcgctgaatcccgcggacgacccgtctcggggccgcttggggccctgtcgtcctcttctctgcctgccgttccgaccgagcacggggcgcacctctctttacgcggactccccgtctgtgccttctcatctgccggaccgtgtgcacttcgcttcacctctgcacgtcgcatggagaccaccgtgaacgcccaccaaagcttgcccaaggtcttacataagaggactcttggactctctgcaatgtcaacgaccgaccttgaggcatacttcaaagactgtttgtttaacgactgggaggagttgggggaggagattaggttaaaggtctttgtactaggaggctgtaggcataaattggtctgcgcaccagcaccatgcaactttttcacctctgcctaatcatcttttgttcatgtcctactgttcaagcctccaagctgtgccttgggtggctttagggcatggacattgacccttataaagaatttgsagcttctgtgcagttactctcgtttttgcctgttsacttctttccttccgtacgagatcttctagataccgcctcagctctgtatcgggatgctttagagtctcctgagcatttgtcaccgcaccatactgcactcaggcaagcaattctttgctggggagaattaatgactctagctacctgggtgggtactaatttagaagatcaagcatctagggacctagtagtcagttatgtcaacamtaatatgggcctaaagtt

SEQ ID NO: 16 - DNA, 957 bp, Hepatitis B virus
cgcatgcgtggaacctttgtggctcctcttccgatccatactgcggaactcctagccgcttgttttgctcgcagccggtctggagcaaacattattgggactgataactctgttgtcctctcccgcaaatatacatcgtttccatggctgctaggccgtgctgccaactgggtcctgcgcgggacgtcctttgtttacgtcccgtcggcgctgaatcccgcggacgacccttctcggggtcgcttgggactctctcgtccccttctccgtctgccgttccgaccgaccacggggcgcacctctctttacgcggactccccgtctgtgccttctcatctgccggaccgtgtgcacttcgcttcacctctgcacgtcgcatggagaccaccgtgaacgcccaccaattgcccaaggtcttacataagaggactcttggactctctgcaatgtcaacgaccgaccttgaggcatacttcaaagactgtttgtttaaagactgggaggagttgggggaggagattagattaaaggtctttgtactaggaggctgtaggcataaattggtctgcgcaccagcaccatgcaactttttcacctctgcctaatcatctcttgttcatgtcctactgttcaagcctccaagctgtgccttgggtggctttggggcatggacattgacccttataaagaatttggagctaccgtggagttactctcatttttgccttctgacttctttccttcggtacgagatcttctagataccgcctcagctctgtatcgggaagctttagagtctcttgagcattgttcacctcaccatactgcactcaggcaagcaattctttgctggggggaactaatgactctagctacctgggtgggagttaatttggaagatccagcatctagggacctagtagtcagttatgtcaacactaatatgggcctaaagtt

SEQ ID NO: 17 - DNA, 960 bp, Hepatitis B virus
cgcatgcgtggaacctttgtggctcctctgccgatccatactgcggaactcctagccgcttgttttgctcgcagcaggtctggagcraaacttatcgggacggataattctgtcgtcctctcccggaaatatacatcgtttccatggctgctaggctgtgctgccaactggatcctgcgagggacgtcctttgtctacgtcccgtcggcgctgaatcctgcggacgacccgtctcggggtcgcttgggggtctatcgtccccttctccgtctrccgttccagccgwccacggggcgcacctctctttacgcggtctccccgtctgtgccttctcgcctgccggwccgtgtgcacttcgcttcacctctgcacgtcgcatggagaccaccgtgaacgcccaccagatattgcccaaggtcttatataagaggactcttggactctctgcaatgtcaacgaccgaccttgaggcatacttcaaagactgtttgtttaaagactgggaggagttgggggaggagattagattaatgatctttgtactaggaggctgtaggcataaawtggtctgcgtaccagcaccatgcaactttttcacctctgcctaatcatctcgtgttcatgtcctactgttcaagcctccaagctgtgccttgagtggctttaggacatggacattgacccttataaagaatttggagcttctgtggagttactctcgtttttgccttctgacttctttccttcagtaagagatcttctagataccgcctctgctctgtttcgggatgccttagaatctcctgagcattgttcacctcaccatactgcactcaggcaagccattctttgctggggagatgtaatgaatctagctacatgggtgggtgcaaatttggaagatccaacatccagggacctggtagtcggttatgtcaatagtaatatgggcctaaagtt

SEQ ID NO: 18 - DNA, 960 bp, Hepatitis B virus
cgcatgcgtggaacctttgyggctcctctgccgatccatactgcggaactcctggccgcttgttttgctcgcagcaggtctggagcgaaacttattggaacggataattctgtcgttctctcccggaaatatacatcatttccatggctgctaggctgtgctgccaactggatcctgcgagggacgtcctttgtctacgtcccgtcagcgctgaatcctgcggacgacccgtctcggggtcgcttggggatctatcgtccccttctccgtctgccgttccggccgaccacggggcgcacctctctttacgcggtctccccgtctgtgccttctcatctgccggaccgtgtgcacttcgcttcacctctgcacgtcgcatggaaaccaccgtgaacgcccaccaaatcttgcccaaggtcttatataagaggactcttggactctctgcaatgtcaacgaccgaccttgaggcatacttcaaagactgcttgtttaaagactgggaggagttgggggaggagattagattaatgatctttgtactaggaggctgtaggcataaattggtctgcgcaccagcaccatgcaactttttcacctctgcctaatcatctcttgttcatgtcctactgttcaagcctccaagctgtgccttgggtggctttaggacatggacattgacccttataaagaatttggagctwctgtggagttactctcktttttgcctcatgacttctttccttcaataagagatcttctagataccgccacagctctgtatcgggatgccttagaatctcctgagcattgttcacctcaccacacggcactcaggcaagccattctttgctggggggatgtaatgaatctagctacctgggtgggtgtaaatttggaagatccagcatccagggacctggtagtcggttatgtcaatactaatatgggcctaaagtt

SEQ ID NO: 19 - DNA, 960 bp, Hepatitis B virus
cgcatgcgtggaacctttgtggctcctctgccgatccatactgcggaactcctagccgcttgttttgctcgcagcaggtctggagcgaaactcatagggacagataattctgtcgttctctcccggaaatatacatcatttccatggctgctaggctgtgctgccaactggatcctgcgagggacgtcctttgtctacgtcccgtcagcgctgaatcctgcggacgacccctctcggggccgcttgggggtctatcgtccccttctccgtctgccgttccggccgaccacggggcgcacctctctttacgcggtctccccgtctgtgccttctcatctgccggaccgtgtgcacttcgcttcacctctgcacgtcgcatggagaccaccgtgaacgcccaccagatcttgcccaaggtcttacataagaggactcttggactctctgcaatgtcaacgaccgaccttgaggcatacttcaaagactgtttgtttaaagactgggaggagttgggggaggagactagattaatgatctttgtactaggaggctgtaggcataaattggtctgcgcaccagcaccatgcaactttttcacctctgcctaatcatctcttgttcatgtcctactgttcaagcctccaagctgtgccttgggtggctttgggacatggacattgacccttataaagaatttggagctactgtggagttactctcgtttttgccttctgacttctttccttcagtaagagatcttctagataccgcctctgctctgtatcgggatgccttagaatctcctgagcattgttcacctcaccatactgcactcaggcaagccattctttgctggggagaattaatgactctagctacctgggtgggtgtaaatttggaagatccagcatccagggacctagtagtcagttatgtcaatactaatatgggcctaaagtt

SEQ ID NO: 20 - DNA, 960 bp, Hepatitis B virus
cgcatgcgtggaacctttgtggctcctctgccgatccatactgcggaactccttgcagcttgtttcgctcgcagccggtctggagcgaaactcatcggcacagacaactctgttgtcctctctaggaagtacacctccttcccatggctgctcggttgtgctgccaactggatcctacgcgggacgtcctttgtttacgtcccgtcggcgctgaatccagcggacgatccctctcggggtcgcttggggctgtatcgcccccttctccgtctgccgttccagccgacgacgggtcgcacctctctttacgcggcctccccgtctgttccttctcgtctgccggaccgtgtgcacttcgcttcacctctgcacgtcgcatggagaccaccgtgaacgcccctcgaagcttgccaacagtcttacataagcggactcttggactttcaggaaggtcaatcacctggatcgaagaatacatcaaagactgtgtatttaaggactgggaggagctgggggaggagattaggttaaaggtctttgtattaggaggctgtaggcataaattggtctgttcaccagcaccatgcaactttttcacctctgcctaatcatcttttgttcatgtcctactgttcaagcctccaagctgtgccttgggtggctttggggcatggacattgacccttataaagaatttggagcttctgtggaattactctcttttttgccttctgacttcttcccgtcagttcgggacctactcgacaccgcttcagccctctaccgggatgctttagaatcaccagaacattgcacacctaaccataccgctctcaggcaagctatattgtgctggggtgagttaatgactttggcttcctgggtgggcaataacttggaagatcctgctgctagggacctagtggttaactatgtcaatactaacatgggcctaaaaat

SEQ ID NO: 21 - DNA, 960 bp, Hepatitis B virus
cgcatgcgtggaacctttgtggctcctctgccgatccatactgcggaactccttgcagcctgtttcgctcgcagccggtctggagcgaacattatcggcacagacaactctgttgtcctctctaggaagtacacctcctttccatggctgctcggttgtgctgccaactggatcctgcgcgggacgtcctttgtttacgtcccgtcggcgctgaatcccgcggacgacccttcccggggtcgcttggggctgtaccgcccccttcttcgtctgccgttccagccgacgacgggtcgcacctctctttacgcggactccccgtctgttccttctcatctgccggaccgtgtgcacttcgcttcacctctgcacgtcgcatggagaccaccgtgaacgccccctggaatctgccaacagtcttacataagaggactcttggactttcaggacggtcaatgacctggatcgaagaatacatcaaagactgtgtatttaaggactgggaggagctgggggaggagatcaggttaaaggtctttgtactaggaggctgtaggcataaattggtctgttcaccagcaccatgcaactttttcacctctgcctaatcatcttttgttcatgtcccactgttcaagcctccaagctgtgccttgggtggctttggggcatggacattgacccttataaagaatttggagcttctgtggaattgctctcttttttgccttctgatttcttcccgtctgttcgggacctactcgacaccgcttcagccctttaccgggatgctctagagtcaccggaacattgcacccccaatcataccgctctcaggcaagctattttgtgctggggtgagttaatgactttggcttcctgggtgggtaataatttggaagaccctgcagctagggatttagtagttaattatgtcaacactaatatgggcctgaaaat

SEQ ID NO: 22 - DNA, 960 bp, Hepatitis B virus
cgcatgcgtggaacctttgtggctcctctgccgatccatactgcggaactccttgcagcctgtttcgctcgcagccggtctggagcgaacattatcggcacagacaactctgttgtcctctctaggaagtacacctcctttccatggctgctcggttgtgctgccaactggatcctgcgcgggacgtcctttgtttacgtcccgtcggcgctgaatcccgcggacgacccttcccggggtcgcttggggctctaccgcccccttcttcgtctgccgttccagccgacgacgggtcgcacctctctttacgcggactccccgtctgttccttctcatctgccggaccgtgtgcacttcgcttcacctctgcacgtcgcatggagaccaccgtgaacgccccctggaatctgccaacagtcttacataagaggactcttggactttcaggacggtcaatgacctggatcgaagaatacatcaaagactgtgtatttaaggactgggaggagctgggggaggagatcaggttaaaggtctttgtactaggaggctgtaggcataaattggtctgttcaccagcaccatgcaactttttcacctctgcctaatcatcttttgttcatgtcccactgttcaagcctccaagctgtgccttgggtggctttggggcatggacattgacccttataaagaatttggcgcttctgtggaattgctctcttttttgccttctgatttcttcccgtctgttcgggacctactcgacaccgcttcagccctttaccgggatgctctagagtcaccggaacattgcacccccaatcataccgctctcaggcaagctattttgtgctggggtgagttaatgactttggcttcctgggtgggtaataatttggaagaccctgcagctagggatttagtagttaattatgtcaacactaatatgggcctgaaaat

SEQ ID NO: 23 - DNA, 996 bp, Hepatitis B virus
cgcatgcgtggaacctttgtggctcctctgccgatccatactgcggaactcctagctgcttgttttgctcgcagccggtctggagcaaaactcattgggactgacaattctgtcgtcctttctcggaaatatacatcctttccatggctgctaggctgtgctgccaactggatccttcgcgggacgtcctttgtttacgtcccgtcagcgctgaatccagcggacgacccctcccggggccgtttggggctctgtcgcccccttctccgtctgccgttcctgccgaccacggggcgcacctctctttacgcggtctccccgtctgttccttctcatctgccggaccgtgtgcacttcgcttcacctctgcacgttacatggaaaccgccatgaacacctctcatcatctgccaaggcagttatataagaggactcttggactgtttgttatgtcaacaaccggggtggagaaatacttcaaggactgtgtttttgctgagtgggaagaattaggcaatgagtccaggttaatgacctttgtattaggaggctgtaggcataaattggtctgcgcaccagcaccatgtaactttttcacctctgcctaatcatctcttgttcatgtcctactgttcaagcctccaagctgtgccttgggtggctttagggcatggatagaacaactttgccatatggcctttttggcttagacattgacccttataaagaatttggagctactgtggagttgctctcgtttttgccttctgactttttcccgtctgttcgtgatcttctcgacaccgcttcagctttgtaccgggaatccttagagtcctctgatcattgttcgcctcaccatacagcactcaggcaagcaatcctgtgctggggtgagttgatgactctagccacctgggtgggtaataatttggaagatccagcatccagagatttggtggtcaattatgttaatactaatatgggtttaaaaat

SEQ ID NO: 24 - DNA, 996 bp, Hepatitis B virus
cgcatgcgtggaacctttgtggctcctctgccgatccatactgcggaactcctagctgcttgttttgctcgcagccggtctggagcaaaactcattgggactgacaattctgtcgtcctttctcggaaatatacatcctttccatggctgctaggctgtgctgccaactggatccttcgcgggacgtcctttgtttacgtcccgtcagcgctgaatccagcggacgacccctcccggggccgtttggggctctgtcgcccccttctccgtctgccgttcctgccgaccacggggcgcacctctctttacgcggtctccccgtctgttccttctcatctgccggaccgtgtgcacttcgcttcacctctgcacgttacatggaaaccgccatgaacacctctcatcatctaccaaggcagttatataagaggactcttggactgtttgttatgtcaacaaccgggatggagaaatacttcaaggactgtgtttttgctgagtgggaagaattaggcaatgagtccaggttaatgacctttgtattaggaggctgtaggcataaattggtctgcgcaccagcaccatgtaactttttcacctctgcctaatcatctcttgttcatgtcctactgttcaagcctccaagctgtgccttgggtggctttagggcatggatagaacaactttgccatatggcctttttggcttagacattgacccttataaagaatttggagctactgtggagttgctctcgtttttgccttctgactttttcccgtctgttcgtgatcttctcgacaccgcttcagctttgtaccgggaatccttagagtcctctgatcattgttcgcctcaccatacagcactcaggcaagcaattctgtgctggggtgagttgatgactctagctacctgggtgggtaataatttggaagatccagcatccagagatttggtggtcaattatgttaatactaatatgggtttaaaaat

SEQ ID NO: 25 - DNA, 999 bp, Hepatitis B virus
cgcatgcgtggaacctttgtggctcctctgccgatccatactgcggaactcctagctgcttgttttgctcgcagccggtctggagcgaaactcattgggactgacaattctgtcgtcctttctcggaaatatacatcctttccatggctgctaggctgtgctgccaactggatccttcgcgggacgtcctttgtttacgtcccgtcagcgctgaatccagcggacgacccctcccggggccgtttggggctctgtcgcccccttctccgtctgccgttcctgccgaccacggggcgcacctctctttacgcggtctccccgtctgttccttctcatctgccggaccgtgtgcacttcgcttcacctctgcacgttacatggaaaccgccatgaacacctctcatcatctgccaaggcagttatataagaggactcttggactgtttgttatgtcaacaaccggggtggagaaatacttcaaggactggtgtgtttttgctgagtgggaagaattaggcaatgagtccaggttaatgacctttgtattaggaggctgtaggcataaattggtctgcgcaccagcaccaatgcaacttttcacctctgcctaatcatctcttgttcatgtcctactgttcaagcctccaagctgtgccttgggtggctttagggcatggatagaacaactttgccatatggcctttttggcttagacattgacccttataaagaatttggagctactgtggagttgctctcgtttttgccttctgactttttcccgtctgttcgtgatcttctcgacaccgcttcagctttgtaccgggaatccttagagtcctctgatcattgttcgcctcaccatacagcactcaggcaagcaatcctgtgctggggtgagttgatgactctagctacctgggtgggtaataatttggaagatccagcatccagagatttggtggtcaattatgttaatactaatatgggtttaaaaat

SEQ ID NO: 26 - DNA, 960 bp, Hepatitis B virus
cgcatgcgcggaacctttgtggctcctctgccgatccatactgcggaactcctagccgcttgtttcgctcgcagcaggtctggagcggacattatcggcactgacaactccgttgtcctttctcggaagtacacctccttcccatggctgctaggatgtgctgccaactggatcctgcgcgggacgtcctttgtctacgtcccgtcggcgctgaatcctgcggacgacccctctcgtggtcgcttggggctctgccgccctcttctccgcctgccgttccggccgacgacgggtcgcacctctctttacgcggactccccgcctgtgccttctcatctgccggcccgtgtgcacttcgcttcacctctgcacgtcgcatggagaccaccgtgaacgccccttggaacttgccaacaaccttacataagaggactcttggactttcgccccggtcaacgacctggattgaggaatacatcaaagactgtgtatttaaggactgggaggagtcgggggaggagttgaggttaaaggtctttgtattaggaggctgtaggcataaattggtctgttcaccagcaccatgcaactttttcacctctgcctaatcatcttttgttcatgtcccactgttcaagcctccaagctgtgccttgggtggctttggggcatggacattgacccttataaagaatttggagcttctgtggagttactctcatttttgccttctgacttcttcccgtctgtccgggacctactcgacaccgcttcagccctctaccgagatgccttagaatcaccagaacattgcacccccaaccacactgctctcaggcaagctattttgcgctggggtgagttgatgaccttggcttcctgggtgggcaataatttagaggatcctgcagcaagagatctagtagttaattatgtcaatactaacatgggcctaaaaat

SEQ ID NO: 27 - DNA, 960 bp, Hepatitis B virus
cgcatgcgcggaacctttgtggctcctctgccgatccatactgcggaactcctagccgcttgtttcgctcgcagcaggtctggagcggacattatcggcactgacaactccgttgtcctttctcggaagtacacctccttcccatggctgctaggttgtgctgccaactggatcctgcgcgggacgtcctttgtctacgtcccgtcggcgctgaatcctgcggacgacccctctcgtggtcgcttggggctctgccgccctcttctccgcctgtcgttccggccgacgacgggtcgcacctctctttacgcggactccccgcctgtgccttctcatctgccggcccgtgtgcacttcgcttcacctctgcacgtcgcatggagaccaccgtgaacgccccttggaacttgccaacaaccttacataagaggactcttggactttcgccccggtcaacgacctggattgaggaatacatcaaagactgtgtatttaaggactgggaggagtcgggggaggagttgaggttaaaggtctttgtattaggaggctgtaggcataaattggtctgttcaccagcaccatgcaactttttcacctctgcctaatcatcttttgttcatgtcccactgttcaagcctccaagctgtgccttgggtggctttggggcatggacattgacccttataaagaatttggagcttctgtggagttactctcatttttgccttctgacttcttcccgtctgtccgggacctactcgacaccgcttcagccctctaccgagatgccttagaatcaccagaacattgcacccccaaccacactgctctcaggcaagctattttgtgctggggtgagttgatgacattggcttcctgggtgggcaataatttagaggatcctgcagcaagagatctagtagttaattatgtcaatactaacatgggcctaaaaat

SEQ ID NO: 28 - DNA, 960 bp, Hepatitis B virus
cgcatgcgcggaaccttttaggctccgctgccgatccatactgcggaactcctagcagcttgtttcgctcgcagccggtctggagcggacattatcggcactgacaactccgttgtcctttctcggaagtacacctccttcccatggctgctaggctgtgctgccaactggatcctgcgcgggacgtcctttgtctacgtcccgtcggcgctgaatcctgcggacgacccctctcgtggtcgcttggggctatgccgccctcttctccgcctgccgttccggccgacgacgggtcgcacctctctttacgcggactccccacctgtgcctttacatcggccggcccgtgtgcacttcgcttcacctctgcacgtcgcatgggaaccaccgtgaacgccccttggaacttgccaacaaccttatataagaggactcttggactttcgccccggtcaacgacctggattgaggaatacatcaaagactgtgtatttaaggactgggaggagtcgggggaggagtcgaggttaatgatctttgtattaggaggctgtaggcataaattggtctgttcaccagcaccatgcaactttttcacctctgcctaatcagcttttgttcatgtcctactgttcaagcctccaagctgtgccttgggtggctttgggacatggacatcgacccttataaagaatttggagcttctgtggagttactctcmtttttgccttctgatttcttcccgtctgtccgggacctactcgacaccgcttcagccctcttccgagatgccttagaatcacccgaacattgcaccccccaccayacagctctcaggcaagctattttgtgctggggtgagttgatgactttggcttcctgggtgggcaataatttagatgatcctgcatccagagatctagtagttaattatgtcaatactaacatgggcctaaaact

SEQ ID NO: 29 - DNA, 960 bp, Hepatitis B virus
cgcatgcgtggaacctttgcagctccactgccgatccatactgcggaactgctagctgcctgttttgctcgcagccggtctggagcaaaacttatcgggactgataattctgtcgtcctttcacggaaatatacatcatttccatggctgctaggctgtgctgccaactggatcatgcgcgggacgtcctttgtctacgtcccgtcggcgctgaatcctgcggacgacccctctcggggccgtttggggatctaccgtccccttctccgtctgccgtaccggccgtccacggggcgcacctctctttacgcggactccccgtgtgtgccttctcatctgccggaccgtgtgcacttcgcttcacctctgcacgtcgcatggagaccaccgtgaacgcccacctggtattgcccaaggtattgcataagaggactcttggactctcggcaatgtcaacgaccgaccttgaggcatacttcaaagactgtgtgtttaaagactgggaggagctgggggaggagattaggctaaaggtctttgtactaggaggctgtaggcataaattggtctgttcaccagcaccatgcaactttttcacctctgcctaatcatctcatgttcatgtcctactgttcaagcctccaagctgtgccttgggtggctttggggcatggacattgacccttataaagaatttggagcttctgtggagttactctcttttttgccttctgatttctctccgtctgttcgagatctactcgacaccgcctcagctctctaccgggaggccttagagtctccggaacattgttcacctcaccatacagcacttaggcaagctgtcctgtgttggggtgagttgatgactctagctacctgggtgggaagtaatttggacgaccctggatccagggatttagtagtcacctatgtcaatgttaatatgggcctaaagtt

SEQ ID NO: 30 - DNA, 960 bp, Hepatitis B virus
cgcatgcgtggaacctttgtggctcctctgccgatccatacggcggaactgctagctgcctgttttgctcgcagcaggtctggggcaaatcttatcgggactgataattctgtcgtcctttcgcggaaatatacatcatttccatggctgctaggctgtgctgccaactggatcctgcgcgggacgtcctttgtctacgtcccgtcggcgctgaatcctgcggacgacccctctcggggccgcttggggatctaccgtccccttcttcgcctgccgttccggccgtccacggggcgcacctctctttacgcggtctccccgtctgtgccttctcatctgccggaccgtgtgcacttcgcttcacctctgcacgtcgcatggagaccaccgtgaacgaccacctgaccttgcccaaggtcttgcataagaggactcttggactcccagcaatgtcaacgaccgaccttgaggcatacttcaaagactgtgtgtttaaagactgggaggagttgggggaggagatcaggttaaagatttatgtattaggaggctgtaggcataaattggtctgcgcaccagcaccatgcaactttttcacctctgcctaatcatctcttgttcatgtcctactgttcaagcctccaagctgtgccttgggtggctttaggacatggacattgacccttataaagaatttggagcttctttggagttactctcttttttgccttctgatttctttccatctgttcgagatctcctcgacaccgcctcagctttgtatcgggaggccttagagtctcctgaacattgtacacctcaccatacagcactcaggcaagcggtaatatgttggggtgagttgatgactctagctacttgggtgggaagtaatttggaagaccctgcctccagggatttagtagtcagctatgtcaatggtcatatgggcctaaaatt

SEQ ID NO: 31 - DNA, 960 bp, Hepatitis B virus
cgcatgcgtggaacctttgtggctcctctgccgatccatactgcggaactgctagctgcctgttttgctcgcagcaggtctggagcaaacattatagggactgataattccgtcgtcctttcgcggaaatatacgtcctttccatggctgctaggctgtgctgccaactggatcctgcgcgggacgtcctttgtctacgtcccgtcggcgctgaatcctgcggacgacccctctcggggccgcttggggatctaccgtccccttcttcgtctgccgttccggccgtccacggggcgcacctctctttacgcggtctccccgtctgtgccttctcatctgccggcccgtgtgcacttcgcttcacctctgcacgtcgcatggagaccaccgtgaacgcccacctgaccttgcccaaggtattgcataagaggactcttggactctcagcaatgtcaacgaccgaccttgaggcatacttcaaagactgtgtgtttaaagactgggaggagttgggggaggagatcaggttaaaggtctttgtattaggaggctgtaggcataaattggtctgttcaccagcaccatgcaactttttcacctctgcctaatcatctcatgttcatgtcctactgttcaagcctccaagttgtgccttgggtggctttggggcatggacattgacccttataaagaatttggagcttctgtggagttactctcttttttgccttctgatttctttccatctattcgagatctcctcgacaccgcctcagctttgtatcgggaggccttagagtctcctgaacattgttcacctcaccatacagcactcaggcaagctgttctatgttggggtgagttgatgactctagctacctgggtgggaagtaatttggaagaccctgcctccagggatttagtagtcagctatgtcaatgttaatatggggctaaaaat

SEQ ID NO: 32 - DNA, 960 bp, Hepatitis B virus
cgcatgcgtggaacctttgtggctcctctgccgatccatactgcggaactcctagcagcttgttttgctcgcagcaggtctggggcaaacctactcgggacagataattctgtggttttatcacggaagtatacgtccttcccatggctgctaggctgtgctgccaactggatcctgcgcgggacgtcctttgtctacgtcccgtcggcgctgaatcccgcggacgacccgtctcggggcaagttgggcctctaccgtcctcttctccgtctgccgttccgaccgaccacggggcgcacctctctttacgcggtctccccgtctgtaccttctcatctgccggcccgtgtgcacttcgcttcacctctgcacgttgcatggagaccaccgtgaacgccccctggaatttgccaagagtgttacataagcggactcttggactttcggacatgtcaacgtccgcaattgagacatacttcaaggactgtgtatttaaagactgggaggagtcaggggaggagattaggttaatgatctttgtattaggaggctgtaggcataaattggtctgttcaccagcaccatgcaactttttcacctctgcctaatcatctcttgttcatgtcctactgttcaagcctccaagctgtgccttgggtggctttagggcatggacattgacccttataaagaatttggagcttctgtggagttactctcttttttgccttctgatttctttccgtcaatcagagacctcctcgacaccgcctcagctctataccgagaagccttagagtctccagaacattgctcacctcaccatacagcacttaggcaagctgtgctatgttggggtgagttgatgaatctggctacctgggtgggaagtaatttggaagacccagcatccagggaacttgtagtcagctatgttaacattaatatgggcctaaaaat

SEQ ID NO: 33 - DNA, 378 bp, Homo sapiens
tatcacagattctttttttttaaattaaagtaacatttccaatctactaatgctaatactgtttcgtatttatagctgatttgatggagttggacatggccatggaaccagacagaaaagcggctgttagtcactggcagcaacagtcttacctggactctggaatccattctggtgccactaccacagctccttctctgagtggtaaaggcaatcctgaggaagaggatgtggatacctcccaagtcctgtatgagtgggaacagggattttctcagtccttcactcaagaacaagtagctggtaagagtattatttttcattgccttactgaaagtcagaatgcagttttgagaactaaaaagttagtgtataata

SEQ ID NO: 34 - DNA, 673 bp, Homo sapiens
gtcgcctgcgctgctctccgcatgtcgctggttccccccggccgccctcaaccccagccggacgccgaccccggggaggcccacctggcggaaggagggggcggcggggggcggccgtgcgtcccagggcacgcacaccaggcactgggccaccagcgcgcggaaagccgccgggtccccgcgctgcaccagccgccagccctggggccccaggcgccgcacgaacgtggccagcggcagcacctcgcggtagtggctgcgcagcagggagcgcacggctcggcagcggggagcgcgcggcatcgcgggggtggccggggccagggcttcccacgtgcgcagcaggacgcagcgctgcctgaaactcgcgccgcgaggagagggcggggccgcggaaaggaaggggaggggctgggagggcccggagggggctgggccggggacccgggaggggtcgggacggggcggggtccgcgcggaggaggcggagctggaaggtgaaggggcaggacgggtgcccgggtccccagtccctccgccacgtgggaagcgcggtcctgggcgtctgtgcccgcgaatccactgggagcccggcctggccccgacagcgcagctgctccgggcggacccgggggtctgggccgcgcttccccgcccgcgcgccgctcgcgct

SEQ ID NO: 35 - DNA, 779 bp, Homo sapiens
ggttccttctctgcaggcccaggtgacccagggttggaagtgtctcatgctggatccccacttttcctcttgcagcagccagactgccttccgggtcactgccatggaggagccgcagtcagatcctagcgtcgagccccctctgagtcaggaaacattttcagacctatggaaactgtgagtggatccattggaagggcaggcccaccacccccaccccaaccccagccccctagcagagacctgtgggaagcgaaaattccatgggactgactttctgctcttgtctttcagacttcctgaaaacaacgttctggtaaggacaagggttgggctggggacctggagggctggggacctggagggctggggggctggggggctgaggacctggtcctctgactgctcttttcacccatctacagtcccccttgccgtcccaagcaatggatgatttgatgctgtccccggacgatattgaacaatggttcactgaagacccaggtccagatgaagctcccagaatgccagaggctgctccccccgtggcccctgcaccagcagctcctacaccggcggcccctgcaccagccccctcctggcccctgtcatcttctgtcccttcccagaaaacctaccagggcagctacggtttccgtctgggcttcttgcattctgggacagccaagtctgtgacttgcacggtcagttgccctgaggggctggcttccatgagacttcaatgcctggccgtatccccctgcatttcttttgtttgg

SEQ ID NO: 36 - DNA, 528 bp, Homo sapiens
gctgccgtcttccagttgctttatctgttcacttgtgccctgactttcaactctgtctccttcctcttcctacagtactcccctgccctcaacaagatgttttgccaactggccaagacctgccctgtgcagctgtgggttgattccacacccccgcccggcacccgcgtccgcgccatggccatctacaagcagtcacagcacatgacggaggttgtgaggcgctgcccccaccatgagcgctgctcagatagcgatggtgagcagctggggctggagagacgacagggctggttgcccagggtccccaggcctctgattcctcactgattgctcttaggtctggcccctcctcagcatcttatccgagtggaaggaaatttgcgtgtggagtatttggatgacagaaacacttttcgacatagtgtggtggtgccctatgagccgcctgaggtctggtttgcaactggggtctctgggaggaggggttaagggtggttgtcagtggccctccaggtgagcagtagg

SEQ ID NO: 37 - DNA, 260 bp, Homo sapiens
aaaaaggcctcccctgcttgccacaggtctccccaaggcgcactggcctcatcttgggcctgtgttatctcctaggttggctctgactgtaccaccatccactacaactacatgtgtaacagttcctgcatgggcggcatgaaccggaggcccatcctcaccatcatcacactggaagactccaggtcaggagccacttgccaccctgcacactggcctgctgtgccccagcctctgcttgcctctgacccctgggccca

SEQ ID NO: 38 - DNA, 436 bp, Homo sapiens
cctggttttttaaatgggacaggtaggacctgatttccttactgcctcttgcttctcttttcctatcctgagtagtggtaatctactgggacggaacagctttgaggtgcgtgtttgtgcctgtcctgggagagaccggcgcacagaggaagagaatctccgcaagaaaggggagcctcaccacgagctgcccccagggagcactaagcgagcctggttttttaaatgggacaggtaggacctgatttccttactgcctcttgcttctcttttcctatcctgagtagcactgcccaacaacaccagctcctctccccagccaaagaagaaaccactggatggagaatatttcacccttcaggtactaagtcttgggacctcttatcaagtggaaagtttccagtctaacactcaaaatgccgttttcttcttgact

SEQ ID NO: 39 - DNA, 453 bp, Homo sapiens
cctggttttttaaatgggacaggtaggacctgatttccttactgcctcttgcttctcttttcctatcctgagtagtggtaatctactgggacggaacagctttgaggtgcgtgtttgtgcctgtcctgggagagaccggcgcacagaggaagagaatctccgcaagaaaggggagcctcaccacgagctgcccccagggagcactaagcgaggtaagcaagcaggacaagaagcggtggaggagaccaagggtgcagttatgcctcagattcacttttatcacctttccttgcctctttcctagcactgcccaacaacaccagctcctctccccagccaaagaagaaaccactggatggagaatatttcacccttcaggtactaagtcttgggacctcttatcaagtggaaagtttccagtctaacactcaaaatgccgttttcttcttgact

SEQ ID NO: 40 - DNA, 257 bp, Homo sapiens
caattgtaacttgaaccatcttttaactcaggtactgtgtatatacttacttctccccctcctctgttgctgcagatccgtgggcgtgagcgcttcgagatgttccgagagctgaatgaggccttggaactcaaggatgcccaggctgggaaggagccaggggggagcagggctcactccaggtgagtgacctcagccccttcctggccctactcccctgccttcctaggttggaaagccataggattccattctca

SEQ ID NO: 41 - DNA, 232 bp, Homo sapiens
ttggtcagggaaaaggggcacagaccctctcactcatgtgatgtcatctctcctccctgcttctgtctcctacagccacctgaagtccaaaaagggtcagtctacctcccgccataaaaaactcatgttcaagacagaagggcctgactcagactgacattctccacttcttgttccccactgacagcctcccacccccatctctccctcccctgccattttgggttttggg

SEQ ID NO: 42 - DNA, 120 bp, Lambda phage
ctggtgccgccgcaatggccattaaccgcgttgcttcatccgcgatatcgcagtcggcgtcacaggttgcccgtgagacaaaggtacgccggaaactggtaaaggaaagggccaggctga

SEQ ID NO: 43 - DNA, 120 bp, Lambda phage
acgtgtcggcggagcagattgcgtatgttgctcagttgcagcgttccggcgatgaagccggggcattgcaggcggcgaacgaggccgcaacgaaagggtttgatgaccagacccgccgcc

SEQ ID NO: 44 - DNA, 120 bp, Lambda phage
gccgtggtggctggtctgccgggggacgattcataagttccgctgtgtgccgcatctcaccgggcggcgctttgagcacggtgtgacggactgttacacactgttccgggatgcttatca

SEQ ID NO: 45 - DNA, 120 bp, Lambda phage
catgtaccgggcgatgttattgaaatctgcgatgatgactatgccggtatcagcaccggtggtcgtgtgctggcggtgaacagccagacccggacgctgacgctcgaccgtgaaatcacg

SEQ ID NO: 46 - DNA, 240 bp, Lambda phage
ctggtgccgccgcaatggccattaaccgcgttgcttcatccgcgatatcgcagtcggcgtcacaggttgcccgtgagacaaaggtacgccggaaactggtaaaggaaagggccaggctgaaaagggccacggtcaaaaatccgcaggccagaatcaaagttaaccggggggatttgcccgtaatcaagctgggtaatgcgcgggttgtcctttcgcgccgcaggcgtcgtaaaaaggggc

SEQ ID NO: 47 - DNA, 240 bp, Lambda phage
catgtaccgggcgatgttattgaaatctgcgatgatgactatgccggtatcagcaccggtggtcgtgtgctggcggtgaacagccagacccggacgctgacgctcgaccgtgaaatcacgctgccatcctccggtaccgcgctgataagcctggttgacggaagtggcaatccggtcagcgtggaggttcagtccgtcaccgacggcgtgaaggtaaaagtgagccgtgttcctgacggt

SEQ ID NO: 48 - DNA, 180 bp, Lambda phage
acgtgtcggcggagcagattgcgtatgttgctcagttgcagcgttccggcgatgaagccggggcattgcaggcggcgaacgaggccgcaacgaaagggtttgatgaccagacccgccgcctgaaagagaacatgggcacgctggagacctgggcagacaggactgcgcgggcattcaaat

SEQ ID NO: 49 - DNA, 180 bp, Lambda phage
gccgtggtggctggtctgccgggggacgattcataagttccgctgtgtgccgcatctcaccgggcggcgctttgagcacggtgtgacggactgttacacactgttccgggatgcttatcatctggcggggattgagatgccggactttcatcgtgaggatgactggtggcgtaacggcca

SEQ ID NO: 50 - DNA, 120 bp, Lambda phage
agttatacattctgccatagattatagctaaggcatgtaataattcgtaatcttttagcgtattagcgacccatcgtctttctgatttaataatagatgattcagttaaatatgaaggta

SEQ ID NO: 51 - DNA, 120 bp, Lambda phage
cacacaacaccatatgcatttaagtcgcttgaaattgctataagcagagcatgttgcgccagcatgattaatacagcatttaatacagagccgtgtttattgagtcggtattcagagtct

SEQ ID NO: 52 - DNA, 120 bp, Lambda phage
gctgacagcctgattgcaaaattcaaagaagcgggcggaacggtcagagagattgatgtatgagcagagtcaccgcgattatctccgctctggttatctgcatcatcgtctgcctgtcat

SEQ ID NO: 53 - DNA, 120 bp, Lambda phage
agaaacgaatgctgcagcgtcacaacaatcagccgccacgtctgcctccaccgcggccacgaaagcgtcagaggccgccacttcagcacgagatgcggtggcctcaaaagaggcagcaaa

SEQ ID NO: 54 - DNA, 120 bp, Lambda phage
atcgccgtgctgccggtgtccggcacgctggtcagccggacgcgggcgctgcagccgtactcggggatgaccggttacaacggcattatcgcccgtctgcaacaggctgccagcgatccg

SEQ ID NO: 55 - DNA, 240 bp, Homo sapiens
gaaaagagctaggaaggacaggcaacttggcaaatcaaagccctgggactagggggttaaaatacagcttcccctcttcccacccgccccagtctctgtcccttttgtaggagggacttagagaaggggtgggcttgccctgtccagttaatttctgacctttactcctgccctttgagtttgatgatgctgagtgtacaagcgttttctccctaaagggtgcagctgagctaggcagca

SEQ ID NO: 56 - DNA, 240 bp, Homo sapiens
gattacgagaggtccctgagtcgcctgacgctggacgacatcgaacggttggccagccgcttcctgcaccctgaagtgactgagacaatggagaagggcttctccaaatagaattctcggagcatggggaggtgcccaacgccaggctaccgctgcatgtcgcactaagtgtgttctcctgttgcagttgggctcatcatcgtcatagctggcatgtacctggctctggccaggtgctag